European Patent Application EP 4 394 038 A1, published July 3, 2024. Title: Transaminase Mutant and Application thereof. Applicant: Asymchem Laboratories(Tianjin) Co.,Ltd. The sequence listing filed with the application follows.

SEQUENCE LISTING (9 sequences)

SEQ ID NO: 1 - protein, 459 aa, Chromobacterium violaceum
MQKQRTCSQWRELDAAHHLHPFTDTASLNQAGARVMTRGEGVYLWDCEGNKIIDGMAGLWCVNVGYGRKDFAEAARRQMEELPFYNTFFGTTHPPVVELSSLLAEVTPAGFDRVFYTNSGSESVDTMIRMVRRYWDVQGKPEKKTLIGRWNGYHGSTIGGASLGGMKYMHEQGDLPIPGMAHIEQPWWYKHGKDMTPDEFGVVAARWLEEKILEIGADKVAAFVGEPIQGAGGVIVPPATYWPEIERICRKYDVLLVADEVICGFGRTGEWFGHQHFGFQPDLFTAAKGLSSGYLPLGAVFVGDRVAEGLIAGGDFNHGFTYSGHPVCAAVAHANVAALRDEGIVQRVKDDIGPYMQKRWRETFSRFEHVDDVRGVGMVLAFTLVKNKAKRELFPDFGEIGTLCEDIFFRNNLIMTACGDHIVSAPPLVMTRAEVDEMLAVAERCLEEFEQTLKARGLA

SEQ ID NO: 2 - DNA, 32 bp, Artificial Sequence
  Saturation mutation primer TA-CV-1-V379NDT-R
  misc_feature (16)..(16): h is a, t, or c
  misc_feature (17)..(17): n is a, t, g, or c
agcgtgaacgccagahncataccaacaccgcg

SEQ ID NO: 3 - DNA, 32 bp, Artificial Sequence
  Saturation mutation primer TA-CV-1-V379NDT-F
  misc_feature (16)..(16): n is a, t, g or c
  misc_feature (17)..(17): d is a, t or g
cgcggtgttggtatgndtctggcgttcacgct

SEQ ID NO: 4 - DNA, 32 bp, Artificial Sequence
  Saturation mutation primer TA-CV-1-V379VHG-R
  misc_feature (16)..(16): d is a,t or g
  misc_feature (17)..(17): b is t, g or c
agcgtgaacgccagcdbcataccaacaccgcg

SEQ ID NO: 5 - DNA, 32 bp, Artificial Sequence
  Saturation mutation primer TA-CV-1-V379VHG-F
  misc_feature (16)..(16): v is a, g or c
  misc_feature (17)..(17): h is a, t or c
cgcggtgttggtatgvhgctggcgttcacgct

SEQ ID NO: 6 - DNA, 31 bp, Artificial Sequence
  Saturation mutation primer TA-CV-1-C418NDT-R
  misc_feature (17)..(17): h is a, t or c
  misc_feature (18)..(18): n is a, t, g or c
cacgatgtgatcgccahnggcagtcataatc

SEQ ID NO: 7 - DNA, 31 bp, Artificial Sequence
  Saturation mutation primer TA-CV-1-C418NDT-F
  misc_feature (14)..(14): n is a, t, g or c
  misc_feature (15)..(15): d is a, t or g
gattatgactgccndtggcgatcacatcgtg

SEQ ID NO: 8 - DNA, 31 bp, Artificial Sequence
  Saturation mutation primer TA-CV-1-C418VHG-R
  misc_feature (17)..(17): d is a, t or g
  misc_feature (18)..(18): b is t, g or c
cacgatgtgatcgcccdbggcagtcataatc

SEQ ID NO: 9 - DNA, 31 bp, Artificial Sequence
  Saturation mutation primer TA-CV-1-C418VHG-F
  misc_feature (14)..(14): v is a, g or c
  misc_feature (15)..(15): h is a, t or c
gattatgactgccvhgggcgatcacatcgtg